European Patent Specification EP 3 800 194 B1, published February 1, 2023. Title: Peptide having activities of skin whitening and uses thereof. Applicant: CAREGEN CO., LTD. The sequence listing filed with the application follows.

SEQUENCE LISTING (15 sequences)

SEQ ID NO: 1 - protein, 5 aa, Artificial Sequence
  Peptide having activities of skin whitening
PNRYP

SEQ ID NO: 2 - DNA, 20 bp, Artificial Sequence
  Forward primer for amplifying Rab27a
gaaaatagcgccaagcaccc

SEQ ID NO: 3 - DNA, 20 bp, Artificial Sequence
  Reverse primer for amplifying Rab27a
cctctttcactgccctctgg

SEQ ID NO: 4 - DNA, 20 bp, Artificial Sequence
  Forward primer for amplifying Mlph
acgatgtcaggggcaaacat

SEQ ID NO: 5 - DNA, 20 bp, Artificial Sequence
  Reverse primer for amplifying Mlph
ctcctctgtgtcagcactgg

SEQ ID NO: 6 - DNA, 20 bp, Artificial Sequence
  Forward primer for amplifying myosin VA
ttctacattgtgggcgccat

SEQ ID NO: 7 - DNA, 19 bp, Artificial Sequence
  Reverse primer for amplifying myosin VA
tcctccaggttggtcaatc

SEQ ID NO: 8 - DNA, 21 bp, Artificial Sequence
  Forward primer for amplifying MITF
ccagcctggcgatcatgtcat

SEQ ID NO: 9 - DNA, 20 bp, Artificial Sequence
  Reverse primer for amplifying MITF
ggtctggacaggagttgctg

SEQ ID NO: 10 - DNA, 20 bp, Artificial Sequence
  Forward primer for amplifying tyrosinase
ggccagctttcaggcagagg

SEQ ID NO: 11 - DNA, 20 bp, Artificial Sequence
  Reverse primer for amplifying tyrosinase
tggtgcttcatgggcaaaat

SEQ ID NO: 12 - DNA, 20 bp, Artificial Sequence
  Forward primer for amplifying TRP1
tctgtgaaggtgtgcaggag

SEQ ID NO: 13 - DNA, 20 bp, Artificial Sequence
  Reverse primer for amplifying TRP1
ccgaaacagagtggaaggtt

SEQ ID NO: 14 - DNA, 25 bp, Artificial Sequence
  Forward primer for amplifying GAPDH
ggtgtgaacggatttggccgtattg

SEQ ID NO: 15 - DNA, 25 bp, Artificial Sequence
  Reverse primer for amplifying GAPDH
ccgttgaatttgccgtgagtggagt